European Patent Application EP 4 147 716 A1, published March 15, 2023. Title: Product. Applicant: Samatva Research Corporation. The sequence listing filed with the application follows.

SEQUENCE LISTING (45 sequences)

SEQ ID NO: 1 - protein, 279 aa, Artificial Sequence
  scFv 9
DPIVMIDNDKPITGGGGSGSQVQLQESGPGLVKPSETLSLTCTVSGYSISSGYYWGWIRQPPGKGLEWIGSIYHSGSTYYNPSLKTRVTISVDTSKNQFSLKLSSVTAADTAVYYCARAVVGIVVVPAAGRRAFDIWGQGTMVTVSSGGGGSGGGGSGGGGSGGGGSGGGGSQSALTQPPSASGSPGQSVTISCTGTSSDVGGYNYVSWYQQHPGKAPKLMIYEVSKRPSGVPDRFSGSKSGNTASLTVSGLQAEDEADYYCSSYAGSNNLVFGGGTKV

SEQ ID NO: 2 - protein, 269 aa, Artificial Sequence
  scFv 10
AHIVMVDAYKPTKGGGGSGSEVQLVESGGGLVQPGGSLRLSCAASGITVSSNYMNWVRQAPGKGLEWVSLIYSGGSTYYADSVKGRFTISRDNSKNTLYLQMNSLRAEDTAVYHCARDLVVYGMDVWGQGTTVTVSSGGGGSGGGGSGGGGSGGGGSGGGGSEIVLTQSPGTLSLSPGERATLSCRASQSVSSSYLAWYQQKPGQAPRLLIYGASSRATGIPDRFSGSGSGTDFTLTISRLEPEDFAVYYCQQYGSSPTFGQGTKLEIK

SEQ ID NO: 3 - protein, 270 aa, Artificial Sequence
  scFv 11
KLGDIEFIKVNKGGGGSGSQVQLVESGGGLVKPGGSLRLSCAASGFTFSDYYMSWIRQAPGKGLEWVSYISSSGSTIYYADSVKGRFTISRDNAKNSLYLQMNSLRAEDTAVYYCARDFSHQQLVPSWGQGTLVTVSSGGGGSGGGGSGGGGSGGGGSGGGGSDIQLTQSPSFLSASVGDRVTITCRASQGISSYLAWYQQKPGKAPKLLIYAASTLQSGVPSRFSGSGSGTEFTLTISSLQPEDFATYYCQQLNSYPLTFGGGTKVEIK

SEQ ID NO: 4 - protein, 6 aa, Artificial Sequence
  Histidine affinity tag
HHHHHH

SEQ ID NO: 5 - protein, 227 aa, Artificial Sequence
  Glutathione-S-transferase (GST) solubility tag
SPILGYWKIKGLVQPTRLLLEYLEEKYEEHLYERDEGDKWRNKKFELGLEFPNLPYYIDGDVKLTQSMAIIRYIADKHNMLGGCPKERAEISMLEGAVLDIRYGVSRIAYSKDFETLKVDFLSKLPEMLKMFEDRLCHKTYLNGDHVTHPDFMLYDALDVVLYMDPMCLDAFPKLVCFKKRIEAIPQIDKYLKSSKYIAWPLQGWQATFGGGDHPPKGIEENLYFQS

SEQ ID NO: 6 - protein, 159 aa, Artificial Sequence
  Cellulose binding domain 3(CBM3)
VSGNLKVEFYNSNPSDTTNSINPQFKVTNTGSSAIDLSKLTLRYYYTVDGQKDQTFWCDHAAIIGSNGSYNGITSNVKGTFVKMSSSTNNADTYLEISFTGGTLEPGAHVQIQGRFAKNDWSNYTQSNDYSFKSASQFVEWDQVTAYLNGVLVWGKESR

SEQ ID NO: 7 - protein, 695 aa, Artificial Sequence
  Karunyam 9
MNHKVHHHHHHIEGRHMSPILGYWKIKGLVQPTRLLLEYLEEKYEEHLYERDEGDKWRNKKFELGLEFPNLPYYIDGDVKLTQSMAIIRYIADKHNMLGGCPKERAEISMLEGAVLDIRYGVSRIAYSKDFETLKVDFLSKLPEMLKMFEDRLCHKTYLNGDHVTHPDFMLYDALDVVLYMDPMCLDAFPKLVCFKKRIEAIPQIDKYLKSSKYIAWPLQGWQATFGGGDHPPKGIEENLYFQSHMELGTLEGEFDPIVMIDNDKPITGGGGSGSQVQLQESGPGLVKPSETLSLTCTVSGYSISSGYYWGWIRQPPGKGLEWIGSIYHSGSTYYNPSLKTRVTISVDTSKNQFSLKLSSVTAADTAVYYCARAVVGIVVVPAAGRRAFDIWGQGTMVTVSSGGGGSGGGGSGGGGSGGGGSGGGGSQSALTQPPSASGSPGQSVTISCTGTSSDVGGYNYVSWYQQHPGKAPKLMIYEVSKRPSGVPDRFSGSKSGNTASLTVSGLQAEDEADYYCSSYAGSNNLVFGGGTKVDSVSGNLKVEFYNSNPSDTTNSINPQFKVTNTGSSAIDLSKLTLRYYYTVDGQKDQTFWCDHAAIIGSNGSYNGITSNVKGTFVKMSSSTNNADTYLEISFTGGTLEPGAHVQIQGRFAKNDWSNYTQSNDYSFKSASQFVEWDQVTAYLNGVLVWGKESR

SEQ ID NO: 8 - protein, 685 aa, Artificial Sequence
  Karunyam 10
MNHKVHHHHHHIEGRHMSPILGYWKIKGLVQPTRLLLEYLEEKYEEHLYERDEGDKWRNKKFELGLEFPNLPYYIDGDVKLTQSMAIIRYIADKHNMLGGCPKERAEISMLEGAVLDIRYGVSRIAYSKDFETLKVDFLSKLPEMLKMFEDRLCHKTYLNGDHVTHPDFMLYDALDVVLYMDPMCLDAFPKLVCFKKRIEAIPQIDKYLKSSKYIAWPLQGWQATFGGGDHPPKGIEENLYFQSHMELGTLEGEFAHIVMVDAYKPTKGGGGSGSEVQLVESGGGLVQPGGSLRLSCAASGITVSSNYMNWVRQAPGKGLEWVSLIYSGGSTYYADSVKGRFTISRDNSKNTLYLQMNSLRAEDTAVYHCARDLVVYGMDVWGQGTTVTVSSGGGGSGGGGSGGGGSGGGGSGGGGSEIVLTQSPGTLSLSPGERATLSCRASQSVSSSYLAWYQQKPGQAPRLLIYGASSRATGIPDRFSGSGSGTDFTLTISRLEPEDFAVYYCQQYGSSPTFGQGTKLEIKDSVSGNLKVEFYNSNPSDTTNSINPQFKVTNTGSSAIDLSKLTLRYYYTVDGQKDQTFWCDHAAIIGSNGSYNGITSNVKGTFVKMSSSTNNADTYLEISFTGGTLEPGAHVQIQGRFAKNDWSNYTQSNDYSFKSASQFVEWDQVTAYLNGVLVWGKESR

SEQ ID NO: 9 - protein, 686 aa, Artificial Sequence
  Karunyam 11
MNHKVHHHHHHIEGRHMSPILGYWKIKGLVQPTRLLLEYLEEKYEEHLYERDEGDKWRNKKFELGLEFPNLPYYIDGDVKLTQSMAIIRYIADKHNMLGGCPKERAEISMLEGAVLDIRYGVSRIAYSKDFETLKVDFLSKLPEMLKMFEDRLCHKTYLNGDHVTHPDFMLYDALDVVLYMDPMCLDAFPKLVCFKKRIEAIPQIDKYLKSSKYIAWPLQGWQATFGGGDHPPKGIEENLYFQSHMELGTLEGEFKLGDIEFIKVNKGGGGSGSQVQLVESGGGLVKPGGSLRLSCAASGFTFSDYYMSWIRQAPGKGLEWVSYISSSGSTIYYADSVKGRFTISRDNAKNSLYLQMNSLRAEDTAVYYCARDFSHQQLVPSWGQGTLVTVSSGGGGSGGGGSGGGGSGGGGSGGGGSDIQLTQSPSFLSASVGDRVTITCRASQGISSYLAWYQQKPGKAPKLLIYAASTLQSGVPSRFSGSGSGTEFTLTISSLQPEDFATYYCQQLNSYPLTFGGGTKVEIKDSVSGNLKVEFYNSNPSDTTNSINPQFKVTNTGSSAIDLSKLTLRYYYTVDGQKDQTFWCDHAAIIGSNGSYNGITSNVKGTFVKMSSSTNNADTYLEISFTGGTLEPGAHVQIQGRFAKNDWSNYTQSNDYSFKSASQFVEWDQVTAYLNGVLVWGKESR

SEQ ID NO: 10 - protein, 25 aa, Artificial Sequence
  FR1 of the heavy chain variable domain of scFv 9
QVQLQESGPGLVKPSETLSLTCTVS

SEQ ID NO: 11 - protein, 9 aa, Artificial Sequence
  CDR1 of the heavy chain variable domain of scFv 9
GYSISSGYY

SEQ ID NO: 12 - protein, 17 aa, Artificial Sequence
  FR2 of the heavy chain variable domain of scFv 9
WGWIRQPPGKGLEWIGS

SEQ ID NO: 13 - protein, 7 aa, Artificial Sequence
  CDR2 of the heavy chain variable domain of scFv 9
IYHSGST

SEQ ID NO: 14 - protein, 38 aa, Artificial Sequence
  FR3 of the heavy chain variable domain of scFv 9
YYNPSLKTRVTISVDTSKNQFSLKLSSVTAADTAVYYC

SEQ ID NO: 15 - protein, 21 aa, Artificial Sequence
  CDR3 of the heavy chain variable domain of scFv 9
ARAVVGIVVVPAAGRRAFDIW

SEQ ID NO: 16 - protein, 25 aa, Artificial Sequence
  FR1 of the light chain variable domain of scFv 9
QSALTQPPSASGSPGQSVTISCTGT

SEQ ID NO: 17 - protein, 9 aa, Artificial Sequence
  CDR1 of the light chain variable domain of scFv 9
SSDVGGYNY

SEQ ID NO: 18 - protein, 17 aa, Artificial Sequence
  FR2 of the light chain variable domain of scFv 9
VSWYQQHPGKAPKLMIY

SEQ ID NO: 19 - protein, 3 aa, Artificial Sequence
  CDR2 of the light chain variable domain of scFv 9
EVS

SEQ ID NO: 20 - protein, 36 aa, Artificial Sequence
  FR3 of the light chain variable domain of scFv 9
KRPSGVPDRFSGSKSGNTASLTVSGLQAEDEADYYC

SEQ ID NO: 21 - protein, 18 aa, Artificial Sequence
  CDR3 of the light chain variable domain of scFv 9
SSYAGSNNLVFGGGTKVD

SEQ ID NO: 22 - protein, 25 aa, Artificial Sequence [sequence omitted]

SEQ ID NO: 23 - protein, 8 aa, Artificial Sequence
  CDR1 of the heavy chain variable domain of scFv 10
GITVSSNY

SEQ ID NO: 24 - protein, 17 aa, Artificial Sequence
  FR2 of the heavy chain variable domain of scFv 10
MNWVRQAPGKGLEWVSL

SEQ ID NO: 25 - protein, 8 aa, Artificial Sequence
  CDR2 of the heavy chain variable domain of scFv 10
IYSGGSTY

SEQ ID NO: 26 - protein, 37 aa, Artificial Sequence
  FR3 of the heavy chain variable domain of scFv 10
YADSVKGRFTISRDNSKNTLYLQMNSLRAEDTAVYHC

SEQ ID NO: 27 - protein, 20 aa, Artificial Sequence
  CDR3 of the heavy chain variable domain of scFv 10
ARDLVVYGMDVWGQGTTVTV

SEQ ID NO: 28 - protein, 23 aa, Artificial Sequence
  FR1 of the light chain variable domain of scFv 10
EIVLTQSPGTLSLSPGERATLSC

SEQ ID NO: 29 - protein, 10 aa, Artificial Sequence
  CDR1 of the light chain variable domain of scFv 10
RASQSVSSSY

SEQ ID NO: 30 - protein, 17 aa, Artificial Sequence
  FR2 of the light chain variable domain of scFv 10
LAWYQQKPGQAPRLLIY

SEQ ID NO: 31 - protein, 3 aa, Artificial Sequence
  CDR2 of the light chain variable domain of scFv 10
GAS

SEQ ID NO: 32 - protein, 56 aa, Artificial Sequence
  FR3 of the light chain variable domain of scFv 10
SRATGIPDRFSGSGSGTDFTLTISRLEPEDFAVYYCQQYGSSPTFGQGTKLEIKVD

SEQ ID NO: 33 - protein, 20 aa, Artificial Sequence
  CDR3 of the light chain variable domain of scFv 10
QQYGSSPTFGQGTKLEIKVD

SEQ ID NO: 34 - protein, 25 aa, Artificial Sequence
  FR1 of the heavy chain variable domain of scFv 11
QVQLVESGGGLVKPGGSLRLSCAAS

SEQ ID NO: 35 - protein, 8 aa, Artificial Sequence
  CDR1 of the heavy chain variable domain of scFv 11
GFTFSDYY

SEQ ID NO: 36 - protein, 17 aa, Artificial Sequence
  FR2 of the heavy chain variable domain of scFv 11
MSWIRQAPGKGLEWVSY

SEQ ID NO: 37 - protein, 8 aa, Artificial Sequence
  CDR2 of the heavy chain variable domain of scFv 11
ISSSGSTI

SEQ ID NO: 38 - protein, 38 aa, Artificial Sequence
  FR3 of the heavy chain variable domain of scFv 11
YYADSVKGRFTISRDNAKNSLYLQMNSLRAEDTAVYYC

SEQ ID NO: 39 - protein, 21 aa, Artificial Sequence
  CDR3 of the heavy chain variable domain of scFv 11
ARDFSHQQLVPSWGQGTLVTV

SEQ ID NO: 40 - protein, 26 aa, Artificial Sequence
  FR1 of the light chain variable domain of scFv 11
DIQLTQSPSFLSASVGDRVTITCRAS

SEQ ID NO: 41 - protein, 6 aa, Artificial Sequence
  CDR1 of the light chain variable domain of scFv 11
QGISSY

SEQ ID NO: 42 - protein, 17 aa, Artificial Sequence
  FR2 of the light chain variable domain of scFv 11
LAWYQQKPGKAPKLLIY

SEQ ID NO: 43 - protein, 3 aa, Artificial Sequence
  CDR2 of the light chain variable domain of scFv 11
AAS

SEQ ID NO: 44 - protein, 36 aa, Artificial Sequence
  FR3 of the light chain variable domain of scFv 11
TLQSGVPSRFSGSGSGTEFTLTISSLQPEDFATYYC

SEQ ID NO: 45 - protein, 21 aa, Artificial Sequence
  CDR3 of the light chain variable domain of scFv 11
QQLNSYPLTFGGGTKVEIKVD